European Patent Application EP 4 702 986 A1, published March 4, 2026. Title: POLYPEPTIDE AND USE THEREOF. Applicant: Biocells (Beijing) Biotech Co., Ltd. The sequence listing filed with the application follows.

SEQUENCE LISTING (88 sequences)

SEQ ID NO: 1 - protein, 14 aa, synthetic construct
  MOD_RES 1: note = X is aspartic acid with a succinyl monoacyl modification
XEEAVYFAHLDIIW

SEQ ID NO: 2 - protein, 14 aa, synthetic construct
  MOD_RES 1: note = X is aspartic acid with a succinyl monoacyl modification
XEEAVYFAHKDIIW

SEQ ID NO: 3 - protein, 14 aa, synthetic construct
  MOD_RES 1: note = X is aspartic acid with a fumaryl monoacyl modification
XEEAVYFAHKDIIW

SEQ ID NO: 4 - protein, 14 aa, synthetic construct
  MOD_RES 1: note = X is aspartic acid with a succinyl monoacyl modification
XEEAVYFAHLDVIW

SEQ ID NO: 5 - protein, 14 aa, synthetic construct
  MOD_RES 1: note = X is aspartic acid with a succinyl monoacyl modification
  MOD_RES 12: note = X is 2-aminobutyric acid
XEEAVYFAHLDXIW

SEQ ID NO: 6 - protein, 14 aa, synthetic construct
  MOD_RES 1: note = X is aspartic acid with a fumaryl monoacyl modification
  MOD_RES 10: note = X is lysine with a AEEA-AEEA-gamma E-ODDA modification
XEEAVYFAHXDIIW

SEQ ID NO: 7 - protein, 14 aa, synthetic construct
  MOD_RES 1: note = X is aspartic acid with a succinyl monoacyl modification
XEEAKYFAHLDIIW

SEQ ID NO: 8 - protein, 14 aa, synthetic construct
  MOD_RES 1: note = X is aspartic acid with a succinyl monoacyl modification
XEEEVYFAHKDIIW

SEQ ID NO: 9 - protein, 14 aa, synthetic construct
  MOD_RES 1: note = X is aspartic acid with a succinyl monoacyl modification
  CROSSLNK 2..5: note = Glutamic acid at position 2 is connected to lysine at position 5 via an intrastrand crosslinking
XEEAKYFAHLDIIW

SEQ ID NO: 10 - protein, 14 aa, synthetic construct
  MOD_RES 1: note = X is aspartic acid with a succinyl monoacyl modification
  MOD_RES 5: note = X is 2-aminobutyric acid
  CROSSLNK 2..5: note = Glutamic acid at position 2 is connected to 2-aminobutyric acid at position 5 via an intrastrand crosslinking
XEEAXYFAHLDIIW

SEQ ID NO: 11 - protein, 14 aa, synthetic construct
  MOD_RES 1: note = X is aspartic acid with a succinyl monoacyl modification
  CROSSLNK 4..10: note = Glutamic acid at position 4 is connected to lysine at position 10 via an intrastrand crosslinking
XEEEVYFAHKDIIW

SEQ ID NO: 12 - protein, 14 aa, synthetic construct
  MOD_RES 1: note = X is aspartic acid with a fumaryl monoacyl modification
  MOD_RES 10: note = X is ornithine with an AEEA-AEEA-gamma E-ODDA modification
XEEAVYFAHXDIIW

SEQ ID NO: 13 - protein, 14 aa, synthetic construct
  MOD_RES 1: note = X is aspartic acid with a fumaryl monoacyl modification
XEEEVYFAHKDIIW

SEQ ID NO: 14 - protein, 14 aa, synthetic construct
  MOD_RES 1: note = X is aspartic acid with a succinyl monoacyl modification
  MOD_RES 10: note = X is ornithine
XEEEVYFAHXDIIW

SEQ ID NO: 15 - protein, 14 aa, synthetic construct
  MOD_RES 1: note = X is aspartic acid with a succinyl monoacyl modification
  MOD_RES 10: note = X is lysine with an AEEA-AEEA-gamma E-ODDA modification
XEEEVYFAHXDIIW

SEQ ID NO: 16 - protein, 15 aa, synthetic construct
  MOD_RES 1: note = X is aspartic acid with a succinyl monoacyl modification
  DISULFID 3..6: note = Cysteine at position 3 is connected to cysteine at position 6 via interchain disulfide bonds
XECEECYFAHKDIIW

SEQ ID NO: 17 - protein, 14 aa, synthetic construct
  MOD_RES 1: note = X is aspartic acid with a fumaryl monomethyl monoacyl modification
XEEEVYFAHKDIIW

SEQ ID NO: 18 - protein, 14 aa, synthetic construct
  MOD_RES 1: note = X is aspartic acid with a fumaryl monoacyl modification
  MOD_RES 10: note = X is ornithine
XEEEVYFAHXDIIW

SEQ ID NO: 19 - protein, 14 aa, synthetic construct
  MOD_RES 1: note = X is aspartic acid with a fumaryl monoacyl modification
  MOD_RES 10: note = X is lysine with an AEEA-AEEA-gamma E-ODDA modification
XEEEVYFAHXDIIW

SEQ ID NO: 20 - protein, 14 aa, synthetic construct
  MOD_RES 1: note = X is aspartic acid with a succinyl monoacyl modification
  MOD_RES 10: note = X is ornithine with an AEEA-AEEA-gamma E-ODDA modification
XEEAVYFAHXDIIW

SEQ ID NO: 21 - protein, 14 aa, synthetic construct
  MOD_RES 1: note = X is aspartic acid with a fumaryl monoacyl modification
  MOD_RES 12: note = X is 2-aminobutyric acid
  CROSSLNK 4..8: note = Glutamic acid at position 4 is connected to lysine at position 8 via an intrastrand crosslinking
XEEEVYFKHKDXIW

SEQ ID NO: 22 - protein, 14 aa, synthetic construct
  MOD_RES 1: note = X is aspartic acid with a succinyl monoacyl modification
  MOD_RES 12: note = X is 2-aminobutyric acid
  CROSSLNK 2..5: note = Glutamic acid at position 2 is connected to lysine at position 5 via an intrastrand crosslinking
XEEAKYFAHLDXIW

SEQ ID NO: 23 - protein, 14 aa, synthetic construct
  MOD_RES 1: note = X is aspartic acid with a fumaryl monoacyl modification
  MOD_RES 12: note = X is 2-aminobutyric acid
  CROSSLNK 2..5: note = Glutamic acid at position 2 is connected to lysine at position 5 via an intrastrand crosslinking
XEEAKYFAHLDXIW

SEQ ID NO: 24 - protein, 14 aa, synthetic construct
  MOD_RES 1: note = X is aspartic acid with a fumaryl monomethyl monoacyl modification
  MOD_RES 12: note = X is 2-aminobutyric acid
  CROSSLNK 2..5: note = Glutamic acid at position 2 is connected to lysine at position 5 via an intrastrand crosslinking
XEEAKYFAHLDXIW

SEQ ID NO: 25 - protein, 14 aa, synthetic construct
  MOD_RES 1: note = X is aspartic acid with a fumaryl monoacyl modification
  MOD_RES 4: note = X is lysine with a gamma E-AEEA-AEEA-ODDA modification
XEEXVYFAHLDIIW

SEQ ID NO: 26 - protein, 14 aa, synthetic construct
  MOD_RES 1: note = X is aspartic acid with a fumaryl monoacyl modification
  MOD_RES 5: note = X is lysine with a gamma E-AEEA-AEEA-ODDA modification
XEEAXYFAHLDIIW

SEQ ID NO: 27 - protein, 14 aa, synthetic construct
  MOD_RES 1: note = X is aspartic acid with a fumaryl monoacyl modification
  MOD_RES 8: note = X is lysine with a gamma E-AEEA-AEEA-ODDA modification
XEEAVYFXHLDIIW

SEQ ID NO: 28 - protein, 14 aa, synthetic construct
  MOD_RES 1: note = X is aspartic acid with a fumaryl monoacyl modification
  MOD_RES 10: note = X is lysine with a gamma E-AEEA-AEEA-C18 modification
XEEAVYFAHXDIIW

SEQ ID NO: 29 - protein, 14 aa, synthetic construct
  MOD_RES 1: note = X is aspartic acid with a fumaryl monoacyl modification
  MOD_RES 10: note = X is lysine with a gamma E-AEEA-AEEA-C16 modification
XEEAVYFAHXDIIW

SEQ ID NO: 30 - protein, 14 aa, synthetic construct
  MOD_RES 1: note = X is aspartic acid with a fumaryl monoacyl modification
  MOD_RES 10: note = X is lysine with a gamma E-AEEA-AEEA-C12 modification
XEEAVYFAHXDIIW

SEQ ID NO: 31 - protein, 14 aa, synthetic construct
  MOD_RES 1: note = X is aspartic acid with a fumaryl monoacyl modification
  MOD_RES 10: note = X is lysine with a gamma E-AEEA-AEEA-B modification
XEEAVYFAHXDIIW

SEQ ID NO: 32 - protein, 14 aa, synthetic construct
  MOD_RES 1: note = X is aspartic acid with a succinyl monoacyl modification
  MOD_RES 10: note = X is lysine with a gamma E-AEEA-AEEA-ODDA modification
XEEAVYFAHXDIIW

SEQ ID NO: 33 - protein, 14 aa, synthetic construct
  MOD_RES 1: note = X is aspartic acid with a fumaryl monomethyl monoacyl modification
  MOD_RES 10: note = X is lysine with a gamma E-AEEA-AEEA-ODDA modification
XEEAVYFAHXDIIW

SEQ ID NO: 34 - protein, 14 aa, synthetic construct
  MOD_RES 1: note = X is aspartic acid with a succinyl monoacyl modification
  CROSSLNK 2..5: note = Glutamic acid at position 2 is connected to lysine at position 5 via an intrastrand crosslinking
XEEAKYFAHLDVIW

SEQ ID NO: 35 - protein, 14 aa, synthetic construct
  MOD_RES 1: note = X is aspartic acid with a succinyl monoacyl modification
  MOD_RES 10: note = X is lysine with a gamma E-AEEA-AEEA-ODDA modification
  CROSSLNK 2..5: note = Glutamic acid at position 2 is connected to lysine at position 5 via an intrastrand crosslinking
XEEAKYFAHXDIIW

SEQ ID NO: 36 - protein, 14 aa, synthetic construct
  MOD_RES 1: note = X is aspartic acid with a succinyl monoacyl modification
  MOD_RES 10: note = X is lysine with a gamma E-AEEA-AEEA-ODDA modification
XEEAVYFAHXDVIW

SEQ ID NO: 37 - protein, 14 aa, synthetic construct
  MOD_RES 1: note = X is aspartic acid with a succinyl monoacyl modification
  MOD_RES 10: note = X is lysine with a gamma E-AEEA-AEEA-ODDA modification
  CROSSLNK 2..5: note = Glutamic acid at position 2 is connected to lysine at position 5 via an intrastrand crosslinking
XEEAKYFAHXDVIW

SEQ ID NO: 38 - protein, 14 aa, synthetic construct
  MOD_RES 1: note = X is aspartic acid with a fumaryl monoacyl modification
  MOD_RES 10: note = X is lysine with a gamma E-AEEA-AEEA-ODDA modification
XEEAVYFAHXDIIW

SEQ ID NO: 39 - protein, 14 aa, synthetic construct
  MOD_RES 1: note = X is aspartic acid with a fumaryl monoacyl modification
  MOD_RES 10: note = X is lysine with a CPAK-MPA modification
XEEAVYFAHXDIIW

SEQ ID NO: 40 - protein, 14 aa, synthetic construct
  MOD_RES 1: note = X is aspartic acid with a fumaryl monoacyl modification
  CROSSLNK 2..5: note = Glutamic acid at position 2 is connected to lysine at position 5 via an intrastrand crosslinking
XEEAKYFAHLDVIW

SEQ ID NO: 41 - protein, 14 aa, synthetic construct
  MOD_RES 1: note = X is aspartic acid with a fumaryl monoacyl modification
  MOD_RES 10: note = X is lysine with a gamma E-AEEA-AEEA-ODDA modification
  CROSSLNK 2..5: note = Glutamic acid at position 2 is connected to lysine at position 5 via an intrastrand crosslinking
XEEAKYFAHXDVIW

SEQ ID NO: 42 - protein, 14 aa, synthetic construct
  MOD_RES 1: note = X is aspartic acid with a fumaryl monoacyl modification
  MOD_RES 10: note = X is lysine with a gamma E-AEEA-AEEA-ODDA modification
XEEAVYFAHXDVIW

SEQ ID NO: 43 - protein, 14 aa, synthetic construct
  MOD_RES 1: note = X is aspartic acid with a fumaryl monoacyl modification
  CROSSLNK 2..5: note = Glutamic acid at position 2 is connected to lysine at position 5 via an intrastrand crosslinking
XEEAKYFAHLDIIW

SEQ ID NO: 44 - protein, 14 aa, synthetic construct
  MOD_RES 1: note = X is aspartic acid with a fumaryl monoacyl modification
  MOD_RES 10: note = X is lysine with a gamma E-AEEA-AEEA-ODDA modification
  CROSSLNK 2..5: note = Glutamic acid at position 2 is connected to lysine at position 5 via an intrastrand crosslinking
XEEAKYFAHXDIIW

SEQ ID NO: 45 - protein, 14 aa, synthetic construct
  MOD_RES 1: note = X is aspartic acid with a fumaryl monoacyl modification
  MOD_RES 10: note = X is lysine with a gamma E-AEEA-AEEA-ODDA modification
  MOD_RES 12: note = X is 2-aminobutyric acid
  CROSSLNK 2..5: note = Glutamic acid at position 2 is connected to lysine at position 5 via an intrastrand crosslinking
XEEAKYFAHXDXIW

SEQ ID NO: 46 - protein, 14 aa, synthetic construct
  MOD_RES 1: note = X is aspartic acid with a fumaryl monoacyl modification
XEEAKYFAHLDIIW

SEQ ID NO: 47 - protein, 14 aa, synthetic construct
  MOD_RES 1: note = X is aspartic acid with a fumaryl monoacyl modification
XEEAKYFAHLDVIW

SEQ ID NO: 48 - protein, 14 aa, synthetic construct
  MOD_RES 1: note = X is aspartic acid with a fumaryl monoacyl modification
  MOD_RES 10: note = X is lysine with a gamma E-AEEA-AEEA-ODDA modification
XEEAKYFAHXDIIW

SEQ ID NO: 49 - protein, 14 aa, synthetic construct
  MOD_RES 1: note = X is aspartic acid with a fumaryl monoacyl modification
  MOD_RES 10: note = X is lysine with a gamma E-AEEA-AEEA-ODDA modification
XEEAKYFAHXDVIW

SEQ ID NO: 50 - protein, 14 aa, synthetic construct
  MOD_RES 1: note = X is aspartic acid with a fumaryl monoacyl modification
  MOD_RES 5: note = X is lysine with a gamma E-AEEA-AEEA-ODDA modification
XEEAXYFAHLDIIW

SEQ ID NO: 51 - protein, 14 aa, synthetic construct
  MOD_RES 1: note = X is aspartic acid with a fumaryl monoacyl modification
  MOD_RES 5: note = X is lysine with a gamma E-AEEA-AEEA-ODDA modification
XEEAXYFAHLDVIW

SEQ ID NO: 52 - protein, 14 aa, synthetic construct
  MOD_RES 1: note = X is aspartic acid with a sorbyl monoacyl modification
XEEAVYFAHLDIIW

SEQ ID NO: 53 - protein, 14 aa, synthetic construct
  MOD_RES 1: note = X is aspartic acid with a trans,trans-muconyl monoacyl modification
XEEAVYFAHLDIIW

SEQ ID NO: 54 - protein, 13 aa, synthetic construct
  MOD_RES 1: note = X is aspartic acid with a fumaryl monoacyl modification
  MOD_RES 13: note = X is isoleucine with a 2-amino-3-(naphthalen-2-yl) propanoic modification
XEEAVYFAHKDIX

SEQ ID NO: 55 - protein, 14 aa, synthetic construct
  MOD_RES 1: note = X is aspartic acid with a succinyl monoacyl modification
  MOD_RES 10: note = X is L-2-amino-4-guanidinobutyric acid
XEEAVYFAHXDIIW

SEQ ID NO: 56 - protein, 14 aa, synthetic construct
  MOD_RES 1: note = X is aspartic acid with a fumaryl monoacyl modification
  MOD_RES 10: note = X is ornithine
XEEAVYFAHXDIIW

SEQ ID NO: 57 - protein, 14 aa, synthetic construct
  MOD_RES 1: note = X is aspartic acid with a fumaryl monoacyl modification
  MOD_RES 10: note = X is citrulline
XEEAVYFAHXDIIW

SEQ ID NO: 58 - protein, 9 aa, synthetic construct
  MOD_RES 1: note = X is Suc-DE cyclo (CEAC)Y
XFAHLDIIW

SEQ ID NO: 59 - protein, 14 aa, synthetic construct
  MOD_RES 1: note = X is aspartic acid with a fumaryl monoacyl modification
XEEAVYFAHKDVIW

SEQ ID NO: 60 - protein, 13 aa, synthetic construct
  MOD_RES 1: note = X is aspartic acid with a fumaryl monoacyl modification
  MOD_RES 11: note = X is aspartic acid with a 2-Abu modification
XEEAVYFAHKXIW

SEQ ID NO: 61 - protein, 14 aa, synthetic construct
  MOD_RES 1: note = X is aspartic acid with a succinyl monoacyl modification
  MOD_RES 12: note = X is isoleucine with a N-Me modification
XEEAVYFAHLDXIW

SEQ ID NO: 62 - protein, 14 aa, synthetic construct
  MOD_RES 1: note = X is aspartic acid with a succinyl monoacyl modification
  MOD_RES 10: note = X is leucine with a N-Me modification
XEEAVYFAHXDIIW

SEQ ID NO: 63 - protein, 14 aa, synthetic construct
  MOD_RES 1: note = X is aspartic acid with a succinyl monoacyl modification
  MOD_RES 10: note = X is leucine with a N-Me modification
  MOD_RES 12: note = X is isoleucine with a N-Me modification
XEEAVYFAHXDXIW

SEQ ID NO: 64 - protein, 14 aa, synthetic construct
  MOD_RES 1: note = X is aspartic acid with a fumaryl monoacyl modification
  MOD_RES 10: note = X is leucine with a N-Me modification
XEEAVYFAHXDIIW

SEQ ID NO: 65 - protein, 14 aa, synthetic construct
  MOD_RES 1: note = X is aspartic acid with a fumaryl monoacyl modification
  MOD_RES 10: note = X is leucine with a N-Me modification
  MOD_RES 12: note = X is isoleucine with a N-Me modification
XEEAVYFAHXDXIW

SEQ ID NO: 66 - protein, 14 aa, synthetic construct
  MOD_RES 1: note = X is aspartic acid with a fumaryl monoacyl modification
XEEAVYFAHLDVIW

SEQ ID NO: 67 - protein, 13 aa, synthetic construct
  MOD_RES 1: note = X is aspartic acid with a fumaryl monoacyl modification
  MOD_RES 11: note = X is aspartic acid with a 2-Abu modification
XEEAVYFAHLXIW

SEQ ID NO: 68 - protein, 14 aa, synthetic construct
  MOD_RES 1: note = X is aspartic acid with a fumaryl monoacyl modification
  CROSSLNK 4..8: note = Glutamic acid at position 4 is connected to glutamic acid at position 8 via an intrastrand crosslinking
XEEEVYFEHKDIIW

SEQ ID NO: 69 - protein, 14 aa, synthetic construct
  MOD_RES 1: note = X is aspartic acid with a fumaryl monoacyl modification
  CROSSLNK 4..10: note = Glutamic acid at position 4 is connected to lysine at position 10 via an intrastrand crosslinking
XEEEVYFKHKDIIW

SEQ ID NO: 70 - protein, 14 aa, synthetic construct
  MOD_RES 1: note = X is aspartic acid with a ferulic modification
XEEAVYFAHKDIIW

SEQ ID NO: 71 - protein, 14 aa, synthetic construct
  MOD_RES 1: note = X is aspartic acid with a fumaryl monoacyl modification
  MOD_RES 4: note = X is glutamic acid with a Biotin modification
XEEXVYFAHKDIIW

SEQ ID NO: 72 - protein, 14 aa, synthetic construct
  MOD_RES 1: note = X is aspartic acid with a succinyl monoacyl modification
XEEAVYFAHLDPIW

SEQ ID NO: 73 - protein, 14 aa, synthetic construct
  MOD_RES 1: note = X is aspartic acid with a fumaryl monoacyl modification
  MOD_RES 3: note = X is glutamic acid with a C16 modification
XEXAVYFAHLDIIW

SEQ ID NO: 74 - protein, 14 aa, synthetic construct
  MOD_RES 1: note = X is aspartic acid with a succinyl monoacyl modification
XEEAVYFAHRDIIW

SEQ ID NO: 75 - protein, 14 aa, synthetic construct
  MOD_RES 1: note = X is aspartic acid with a fumaryl monoacyl modification
XEEALYFAHKDIIW

SEQ ID NO: 76 - protein, 14 aa, synthetic construct
  MOD_RES 1: note = X is aspartic acid with a fumaryl monoacyl modification
XEEAFYFAHKDIIW

SEQ ID NO: 77 - protein, 14 aa, synthetic construct
  MOD_RES 1: note = X is aspartic acid with a fumaryl monoacyl modification
  MOD_RES 10: note = X is lysine with an AEEA-gamma E-C18 modification
XEEAVYFAHXDIIW

SEQ ID NO: 78 - protein, 14 aa, synthetic construct
  MOD_RES 1: note = X is aspartic acid with a fumaryl monoacyl modification
  MOD_RES 10: note = X is lysine with an AEEA-gamma E-C16 modification
XEEAVYFAHXDIIW

SEQ ID NO: 79 - protein, 14 aa, synthetic construct
  MOD_RES 1: note = X is aspartic acid with a fumaryl monoacyl modification
  MOD_RES 10: note = X is lysine with an AEEA-gamma E-C12 modification
XEEAVYFAHXDIIW

SEQ ID NO: 80 - protein, 14 aa, synthetic construct
  MOD_RES 1: note = X is lysine with a fumaryl monoacyl modification and an AEEA-AEEA-gamma E -ODDA modification
XEEAVYFAHLDIIW

SEQ ID NO: 81 - protein, 14 aa, synthetic construct
  MOD_RES 1: note = X is aspartic acid with a fumaryl monoacyl modification
  MOD_RES 2: note = X is lysine with an AEEA-AEEA-gamma E-ODDA modification
XXEAVYFAHLDIIW

SEQ ID NO: 82 - protein, 15 aa, synthetic construct
  MOD_RES 1: note = X is aspartic acid with an ODDA-gamma E-AEEA-AEEA modification
XDEEAVYFAHLDIIW

SEQ ID NO: 83 - protein, 14 aa, synthetic construct
  MOD_RES 1: note = X is aspartic acid with an ODDA-gamma E-AEEA-AEEA-NH-C2H4-NH-succinyl monoacyl modification
XEEAVYFAHLDIIW

SEQ ID NO: 84 - protein, 14 aa, synthetic construct
  MOD_RES 1: note = X is 2-(2,5-dioxopyrrolidin-1-yl) succinate
  MOD_RES 10: note = X is lysine with an ODDA-gamma E-AEEA-AEEA modification
XEEAVYFAHXDIIW

SEQ ID NO: 85 - protein, 21 aa, synthetic construct
CSCSSLMDKECVYFCHLDIIW

SEQ ID NO: 86 - protein, 14 aa, synthetic construct
  MOD_RES 1: note = X is aspartic acid with a fumaryl monoacyl modification
  MOD_RES 10: note = X is lysine with an AEEA-gamma E-C12 modification
XEEAVYFAHXDVIW

SEQ ID NO: 87 - protein, 15 aa, synthetic construct
  MOD_RES 1: note = X is aspartic acid with a fumaryl monoacyl modification
  MOD_RES 10: note = X is lysine with an AEEA-E-C12 modification
XDEEAVYFAHXDVIW

SEQ ID NO: 88 - protein, 9 aa, synthetic construct
  MOD_RES 1: note = X is tyrosine with a Suc-DE cyclo (CEEC) modification
XFAHLDIIW